European Patent Application EP 4 343 005 A1, published March 27, 2024. Title: 프로바이오틱스 조성물 내 균종 판별을 위한 프라이머 세트 및 이를 이용한 균종 판별 방법. Applicant: 종근당건강 주식회사. Application KR. The sequence listing filed with the application follows.

SEQUENCE LISTING (18 sequences)

SEQ ID NO: 1 - DNA, 20 bp, synthetic construct
  misc_feature 1..20: note = ITS forward primer
  source 1..20: mol_type = other DNA
tgcggytggatcmcctcctt

SEQ ID NO: 2 - DNA, 18 bp, synthetic construct
  misc_feature 1..18: note = ITS-Lactobacillus reverse primer
  source 1..18: mol_type = other DNA
tccttcatcgrctcctag

SEQ ID NO: 3 - DNA, 19 bp, synthetic construct
  misc_feature 1..19: note = ITS-L. acidophilus reverse primer
  source 1..19: mol_type = other DNA
cgcccttytyyacttgacc

SEQ ID NO: 4 - DNA, 18 bp, synthetic construct
  misc_feature 1..18: note = ITS-Bifidobacterium reverse primer
  source 1..18: mol_type = other DNA
cagttctcaarccaccac

SEQ ID NO: 5 - DNA, 20 bp, synthetic construct
  misc_feature 1..20: note = ITS-coccus reverse primer
  source 1..20: mol_type = other DNA
caatggagcctagcgggatc

SEQ ID NO: 6 - DNA, 18 bp, synthetic construct
  misc_feature 1..18: note = ITS-Enterococcus reverse primer
  source 1..18: mol_type = other DNA
attcaacgcggtgttctc

SEQ ID NO: 7 - DNA, 20 bp, synthetic construct
  misc_feature 1..20: note = ITS-Enterobacteria reverse primer
  source 1..20: mol_type = other DNA
caattttcagcttgatccag

SEQ ID NO: 8 - DNA, 20 bp, synthetic construct
  misc_feature 1..20: note = ITS-Staphylococcus reverse primer
  source 1..20: mol_type = other DNA
gttcttycgaacactagcga

SEQ ID NO: 9 - DNA, 20 bp, synthetic construct
  misc_feature 1..20: note = ITS-Pseudomonas reverse primer
  source 1..20: mol_type = other DNA
ggaggatcgaactcctgacc

SEQ ID NO: 10 - DNA, 53 bp, synthetic construct
  misc_feature 1..53: note = ITS forward illlumina adaptor fusion primer
  source 1..53: mol_type = other DNA
tcgtcggcagcgtcagatgtgtataagagacagtgcggytggatcmcctcctt

SEQ ID NO: 11 - DNA, 52 bp, synthetic construct
  misc_feature 1..52: note = ITS-Lactobacillus reverse illumina adaptor fusion primer
  source 1..52: mol_type = other DNA
gtctcgtgggctcggagatgtgtataagagacagtccttcatcgrctcctag

SEQ ID NO: 12 - DNA, 53 bp, synthetic construct
  misc_feature 1..53: note = ITS-L. acidophilus reverse illumina adaptor fusion primer
  source 1..53: mol_type = other DNA
gtctcgtgggctcggagatgtgtataagagacagcgcccttytyyacttgacc

SEQ ID NO: 13 - DNA, 52 bp, synthetic construct
  misc_feature 1..52: note = ITS-Bifidobacterium reverse illumina adaptor fusion primer
  source 1..52: mol_type = other DNA
gtctcgtgggctcggagatgtgtataagagacagcagttctcaarccaccac

SEQ ID NO: 14 - DNA, 54 bp, synthetic construct
  misc_feature 1..54: note = ITS-coccus reverse illumina adaptor fusion primer
  source 1..54: mol_type = other DNA
gtctcgtgggctcggagatgtgtataagagacagcaatggagcctagcgggatc

SEQ ID NO: 15 - DNA, 52 bp, synthetic construct
  misc_feature 1..52: note = ITS-Enterococcus reverse illumina adaptor fusion primer
  source 1..52: mol_type = other DNA
gtctcgtgggctcggagatgtgtataagagacagattcaacgcggtgttctc

SEQ ID NO: 16 - DNA, 54 bp, synthetic construct
  misc_feature 1..54: note = ITS-Enterobacteria reverse illumina adaptor fusion primer
  source 1..54: mol_type = other DNA
gtctcgtgggctcggagatgtgtataagagacagcaattttcagcttgatccag

SEQ ID NO: 17 - DNA, 54 bp, synthetic construct
  misc_feature 1..54: note = ITS-Staphylococcus reverse illumina adaptor fusion primer
  source 1..54: mol_type = other DNA
gtctcgtgggctcggagatgtgtataagagacaggttcttycgaacactagcga

SEQ ID NO: 18 - DNA, 54 bp, synthetic construct
  misc_feature 1..54: note = ITS-Pseudomonas reverse illumina adaptor fusion primer
  source 1..54: mol_type = other DNA
gtctcgtgggctcggagatgtgtataagagacagggaggatcgaactcctgacc